European Patent Specification EP 3 411 058 B1, published March 8, 2023. Title: COMBINATION THERAPY WITH A6, CHEMOTHERAPEUTIC AGENTS, RADIATION THERAPY, OR A COMBINATION THEREOF FOR THE TREATMENT OF CANCER. Applicant: Splash Pharmaceuticals, Inc. The sequence listing filed with the application follows.

SEQUENCE LISTING (6 sequences)

SEQ ID NO: 1 - protein, 8 aa, Artificial Sequence
  A6
  MOD_RES (1)..(1): ACETYLATION
  MOD_RES (8)..(8): AMIDATION
KPSSPPEE

SEQ ID NO: 2 - protein, 8 aa, Artificial Sequence
  CD44 Sequence Homolog
  MOD_RES (1)..(1): ACETYLATION
  MOD_RES (8)..(8): AMIDATION
NASAPPEE

SEQ ID NO: 3 - protein, 14 aa, Artificial Sequence
  CD44-modulating polypeptide 3
QETWFQNGWQGKNP

SEQ ID NO: 4 - protein, 14 aa, Artificial Sequence
  CD44-modulating polypeptide 4
KEKWFENEWQGKNP

SEQ ID NO: 5 - protein, 14 aa, Artificial Sequence
  CD44-modulating polypeptide 5
KEQWFGNRWHEGYR

SEQ ID NO: 6 - protein, 24 aa, Artificial Sequence
  CD44-modulating polypeptide 6
QIRQQPRDPPTETLELEVSPDPAS